European Patent Application EP 4 215 542 A1, published July 26, 2023. Title: IL-2 mutant protein and drugs containing it. Applicant: MIYAGI PREFECTURAL HOSPITAL ORGANIZATION. The sequence listing filed with the application follows.

SEQUENCE LISTING (33 sequences)

SEQ ID NO: 1 - protein, 133 aa, Homo sapiens [sequence omitted]

SEQ ID NO: 2 - protein, 133 aa, Artificial Sequence
  Aldesleukin
APASSSTKKTQLQLEHLLLDLQMILNGINNYKNPKLTRMLTFKFYMPKKATELKHLQCLEEELKPLEEVLNLAQSKNFHLRPRDLISNINVIVLELKGSETTFMCEYADETATIVEFLNRWITFAQSIISTLT

SEQ ID NO: 3 - protein, 133 aa, Artificial Sequence
  MK-6-IL-2
APASSSTKKTQLQLEHLLLDLQMILNGINNYKNPALTAMLTFAFAMPKKATELKHLQCLEEELKPLEEVLNLAQSKNFHLRPRDLISNINVIVLELKGSETTFMCEYADETATIVEFLNRWITFAQSIISTLT

SEQ ID NO: 4 - protein, 133 aa, Artificial Sequence
  MK-15-IL-2
APASSSTKKTQLQLEHLLLDLQMILNGINNYKNPALTAMLTAKFAMPKKATELKHLQCLEEELKPLEEVLNLAQSKNFHLRPRDLISNINVIVLELKGSETTFMCEYADETATIVEFLNRWITFAQSIISTLT

SEQ ID NO: 5 - protein, 133 aa, Artificial Sequence
  MK-4-IL-2
APASSSTKKTQLQLEHLLLDLQMILNGINNYKNPALTAMLTFKFYMPKKATELKHLQCLEEELKPLEEVLNLAQSKNFHLRPRDLISNINVIVLELKGSETTFMCEYADETATIVEFLNRWITFAQSIISTLT

SEQ ID NO: 6 - protein, 585 aa, Homo sapiens [sequence omitted]

SEQ ID NO: 7 - protein, 733 aa, Artificial Sequence
  HSA-3xG4S-MK-6
DAHKSEVAHRFKDLGEENFKALVLIAFAQYLQQCPFEDHVKLVNEVTEFAKTCVADESAENCDKSLHTLFGDKLCTVATLRETYGEMADCCAKQEPERNECFLQHKDDNPNLPRLVRPEVDVMCTAFHDNEETFLKKYLYEIARRHPYFYAPELLFFAKRYKAAFTECCQAADKAACLLPKLDELRDEGKASSAKQRLKCASLQKFGERAFKAWAVARLSQRFPKAEFAEVSKLVTDLTKVHTECCHGDLLECADDRADLAKYICENQDSISSKLKECCEKPLLEKSHCIAEVENDEMPADLPSLAADFVESKDVCKNYAEAKDVFLGMFLYEYARRHPDYSVVLLLRLAKTYETTLEKCCAAADPHECYAKVFDEFKPLVEEPQNLIKQNCELFEQLGEYKFQNALLVRYTKKVPQVSTPTLVEVSRNLGKVGSKCCKHPEAKRMPCAEDYLSVVLNQLCVLHEKTPVSDRVTKCCTESLVNRRPCFSALEVDETYVPKEFNAETFTFHADICTLSEKERQIKKQTALVELVKHKPKATKEQLKAVMDDFAAFVEKCCKADDKETCFAEEGKKLVAASQAALGLGGGGSGGGGSGGGGSAPASSSTKKTQLQLEHLLLDLQMILNGINNYKNPALTAMLTFAFAMPKKATELKHLQCLEEELKPLEEVLNLAQSKNFHLRPRDLISNINVIVLELKGSETTFMCEYADETATIVEFLNRWITFAQSIISTLT

SEQ ID NO: 8 - protein, 733 aa, Artificial Sequence
  HSA-3xG4S-MK-15
DAHKSEVAHRFKDLGEENFKALVLIAFAQYLQQCPFEDHVKLVNEVTEFAKTCVADESAENCDKSLHTLFGDKLCTVATLRETYGEMADCCAKQEPERNECFLQHKDDNPNLPRLVRPEVDVMCTAFHDNEETFLKKYLYEIARRHPYFYAPELLFFAKRYKAAFTECCQAADKAACLLPKLDELRDEGKASSAKQRLKCASLQKFGERAFKAWAVARLSQRFPKAEFAEVSKLVTDLTKVHTECCHGDLLECADDRADLAKYICENQDSISSKLKECCEKPLLEKSHCIAEVENDEMPADLPSLAADFVESKDVCKNYAEAKDVFLGMFLYEYARRHPDYSVVLLLRLAKTYETTLEKCCAAADPHECYAKVFDEFKPLVEEPQNLIKQNCELFEQLGEYKFQNALLVRYTKKVPQVSTPTLVEVSRNLGKVGSKCCKHPEAKRMPCAEDYLSVVLNQLCVLHEKTPVSDRVTKCCTESLVNRRPCFSALEVDETYVPKEFNAETFTFHADICTLSEKERQIKKQTALVELVKHKPKATKEQLKAVMDDFAAFVEKCCKADDKETCFAEEGKKLVAASQAALGLGGGGSGGGGSGGGGSAPASSSTKKTQLQLEHLLLDLQMILNGINNYKNPALTAMLTAKFAMPKKATELKHLQCLEEELKPLEEVLNLAQSKNFHLRPRDLISNINVIVLELKGSETTFMCEYADETATIVEFLNRWITFAQSIISTLT

SEQ ID NO: 9 - protein, 733 aa, Artificial Sequence
  HSA-3x(EAAAK)-MK-6
DAHKSEVAHRFKDLGEENFKALVLIAFAQYLQQCPFEDHVKLVNEVTEFAKTCVADESAENCDKSLHTLFGDKLCTVATLRETYGEMADCCAKQEPERNECFLQHKDDNPNLPRLVRPEVDVMCTAFHDNEETFLKKYLYEIARRHPYFYAPELLFFAKRYKAAFTECCQAADKAACLLPKLDELRDEGKASSAKQRLKCASLQKFGERAFKAWAVARLSQRFPKAEFAEVSKLVTDLTKVHTECCHGDLLECADDRADLAKYICENQDSISSKLKECCEKPLLEKSHCIAEVENDEMPADLPSLAADFVESKDVCKNYAEAKDVFLGMFLYEYARRHPDYSVVLLLRLAKTYETTLEKCCAAADPHECYAKVFDEFKPLVEEPQNLIKQNCELFEQLGEYKFQNALLVRYTKKVPQVSTPTLVEVSRNLGKVGSKCCKHPEAKRMPCAEDYLSVVLNQLCVLHEKTPVSDRVTKCCTESLVNRRPCFSALEVDETYVPKEFNAETFTFHADICTLSEKERQIKKQTALVELVKHKPKATKEQLKAVMDDFAAFVEKCCKADDKETCFAEEGKKLVAASQAALGLEAAAKEAAAKEAAAKAPASSSTKKTQLQLEHLLLDLQMILNGINNYKNPALTAMLTFAFAMPKKATELKHLQCLEEELKPLEEVLNLAQSKNFHLRPRDLISNINVIVLELKGSETTFMCEYADETATIVEFLNRWITFAQSIISTLT

SEQ ID NO: 10 - protein, 733 aa, Artificial Sequence
  HSA-3x(EAAAK)-MK-15
DAHKSEVAHRFKDLGEENFKALVLIAFAQYLQQCPFEDHVKLVNEVTEFAKTCVADESAENCDKSLHTLFGDKLCTVATLRETYGEMADCCAKQEPERNECFLQHKDDNPNLPRLVRPEVDVMCTAFHDNEETFLKKYLYEIARRHPYFYAPELLFFAKRYKAAFTECCQAADKAACLLPKLDELRDEGKASSAKQRLKCASLQKFGERAFKAWAVARLSQRFPKAEFAEVSKLVTDLTKVHTECCHGDLLECADDRADLAKYICENQDSISSKLKECCEKPLLEKSHCIAEVENDEMPADLPSLAADFVESKDVCKNYAEAKDVFLGMFLYEYARRHPDYSVVLLLRLAKTYETTLEKCCAAADPHECYAKVFDEFKPLVEEPQNLIKQNCELFEQLGEYKFQNALLVRYTKKVPQVSTPTLVEVSRNLGKVGSKCCKHPEAKRMPCAEDYLSVVLNQLCVLHEKTPVSDRVTKCCTESLVNRRPCFSALEVDETYVPKEFNAETFTFHADICTLSEKERQIKKQTALVELVKHKPKATKEQLKAVMDDFAAFVEKCCKADDKETCFAEEGKKLVAASQAALGLEAAAKEAAAKEAAAKAPASSSTKKTQLQLEHLLLDLQMILNGINNYKNPALTAMLTAKFAMPKKATELKHLQCLEEELKPLEEVLNLAQSKNFHLRPRDLISNINVIVLELKGSETTFMCEYADETATIVEFLNRWITFAQSIISTLT

SEQ ID NO: 11 - protein, 584 aa, Mus musculus
EAHKSEIAHRYNDLGEQHFKGLVLIAFSQYLQKCSYDEHAKLVQEVTDFAKTCVADESAANCDKSLHTLFGDKLCAIPNLRENYGELADCCTKQEPERNECFLQHKDDNPSLPPFERPEAEAMCTSFKENPTTFMGHYLHEVARRHPYFYAPELLYYAEQYNEILTQCCAEADKESCLTPKLDGVKEKALVSSVRQRMKCSSMQKFGERAFKAWAVARLSQTFPNADFAEITKLATDLTKVNKECCHGDLLECADDRAELAKYMCENQATISSKLQTCCDKPLLKKAHCLSEVEHDTMPADLPAIAADFVEDQEVCKNYAEAKDVFLGTFLYEYSRRHPDYSVSLLLRLAKKYEATLEKCCAEANPPACYGTVLAEFQPLVEEPKNLVKTNCDLYEKLGEYGFQNAILVRYTQKAPQVSTPTLVEAARNLGRVGTKCCTLPEDQRLPCVEDYLSAILNRVCLLHEKTPVSEHVTKCCSGSLVERRPCFSALTVDETYVPKEFKAETFTFHSDICTLPEKEKQIKKQTALAELVKHKPKATAEQLKTVMDDFAQFLDTCCKAADKDTCFSTEGPNLVTRCKDALA

SEQ ID NO: 12 - protein, 732 aa, Artificial Sequence
  MSA-MK-6
APASSSTKKTQLQLEHLLLDLQMILNGINNYKNPALTAMLTFAFAMPKKATELKHLQCLEEELKPLEEVLNLAQSKNFHLRPRDLISNINVIVLELKGSETTFMCEYADETATIVEFLNRWITFAQSIISTLTGGGGSGGGGSGGGGSEAHKSEIAHRYNDLGEQHFKGLVLIAFSQYLQKCSYDEHAKLVQEVTDFAKTCVADESAANCDKSLHTLFGDKLCAIPNLRENYGELADCCTKQEPERNECFLQHKDDNPSLPPFERPEAEAMCTSFKENPTTFMGHYLHEVARRHPYFYAPELLYYAEQYNEILTQCCAEADKESCLTPKLDGVKEKALVSSVRQRMKCSSMQKFGERAFKAWAVARLSQTFPNADFAEITKLATDLTKVNKECCHGDLLECADDRAELAKYMCENQATISSKLQTCCDKPLLKKAHCLSEVEHDTMPADLPAIAADFVEDQEVCKNYAEAKDVFLGTFLYEYSRRHPDYSVSLLLRLAKKYEATLEKCCAEANPPACYGTVLAEFQPLVEEPKNLVKTNCDLYEKLGEYGFQNAILVRYTQKAPQVSTPTLVEAARNLGRVGTKCCTLPEDQRLPCVEDYLSAILNRVCLLHEKTPVSEHVTKCCSGSLVERRPCFSALTVDETYVPKEFKAETFTFHSDICTLPEKEKQIKKQTALAELVKHKPKATAEQLKTVMDDFAQFLDTCCKAADKDTCFSTEGPNLVTRCKDALA

SEQ ID NO: 13 - protein, 732 aa, Artificial Sequence
  MSA-MK-14
APASSSTKKTQLQLEHLLLDLQMILNGINNYKNPKLTRMLTFKFYMPKKATELKHLQCLEEELKPLEEVLNLAQSKNFHLRPRDLISNINVIVLELKGSETTFMCEYADETATIVEFLNRWITFAQSIISTLTGGGGSGGGGSGGGGSEAHKSEIAHRYNDLGEQHFKGLVLIAFSQYLQKCSYDEHAKLVQEVTDFAKTCVADESAANCDKSLHTLFGDKLCAIPNLRENYGELADCCTKQEPERNECFLQHKDDNPSLPPFERPEAEAMCTSFKENPTTFMGHYLHEVARRHPYFYAPELLYYAEQYNEILTQCCAEADKESCLTPKLDGVKEKALVSSVRQRMKCSSMQKFGERAFKAWAVARLSQTFPNADFAEITKLATDLTKVNKECCHGDLLECADDRAELAKYMCENQATISSKLQTCCDKPLLKKAHCLSEVEHDTMPADLPAIAADFVEDQEVCKNYAEAKDVFLGTFLYEYSRRHPDYSVSLLLRLAKKYEATLEKCCAEANPPACYGTVLAEFQPLVEEPKNLVKTNCDLYEKLGEYGFQNAILVRYTQKAPQVSTPTLVEAARNLGRVGTKCCTLPEDQRLPCVEDYLSAILNRVCLLHEKTPVSEHVTKCCSGSLVERRPCFSALTVDETYVPKEFKAETFTFHSDICTLPEKEKQIKKQTALAELVKHKPKATAEQLKTVMDDFAQFLDTCCKAADKDTCFSTEGPNLVTRCKDALA

SEQ ID NO: 14 - protein, 732 aa, Artificial Sequence
  MSA-MK-15
APASSSTKKTQLQLEHLLLDLQMILNGINNYKNPALTAMLTAKFAMPKKATELKHLQCLEEELKPLEEVLNLAQSKNFHLRPRDLISNINVIVLELKGSETTFMCEYADETATIVEFLNRWITFAQSIISTLTGGGGSGGGGSGGGGSEAHKSEIAHRYNDLGEQHFKGLVLIAFSQYLQKCSYDEHAKLVQEVTDFAKTCVADESAANCDKSLHTLFGDKLCAIPNLRENYGELADCCTKQEPERNECFLQHKDDNPSLPPFERPEAEAMCTSFKENPTTFMGHYLHEVARRHPYFYAPELLYYAEQYNEILTQCCAEADKESCLTPKLDGVKEKALVSSVRQRMKCSSMQKFGERAFKAWAVARLSQTFPNADFAEITKLATDLTKVNKECCHGDLLECADDRAELAKYMCENQATISSKLQTCCDKPLLKKAHCLSEVEHDTMPADLPAIAADFVEDQEVCKNYAEAKDVFLGTFLYEYSRRHPDYSVSLLLRLAKKYEATLEKCCAEANPPACYGTVLAEFQPLVEEPKNLVKTNCDLYEKLGEYGFQNAILVRYTQKAPQVSTPTLVEAARNLGRVGTKCCTLPEDQRLPCVEDYLSAILNRVCLLHEKTPVSEHVTKCCSGSLVERRPCFSALTVDETYVPKEFKAETFTFHSDICTLPEKEKQIKKQTALAELVKHKPKATAEQLKTVMDDFAQFLDTCCKAADKDTCFSTEGPNLVTRCKDALA

SEQ ID NO: 15 - protein, 251 aa, Artificial Sequence
  Human anti CSPG4-scFv
EAQLVESGAEVKKPGDSLKISCKGSGYSFTSYWIGWVRQMPGKGLEWMGIIYPGDSETTYSPAFQGDVTISVDKSISTAYLQWNSLKASDTGIYYCARRRGNYYMDVWGNGTPVTVSSLKSGGGGSGGGGSGGGGSRSTQSALTQPASVSGSPGQSITISCTGTSSDVGGYNYVSWYQQHPGKAPKLMIYDVSNRPSGVSNRFSGSKSGNTASLTISGLQAEDEADYYCSSYTSSSTRHVFGTGTQLTVLG

SEQ ID NO: 16 - protein, 999 aa, Artificial Sequence
  HSA-CSPG4-scFv-MK-6
DAHKSEVAHRFKDLGEENFKALVLIAFAQYLQQCPFEDHVKLVNEVTEFAKTCVADESAENCDKSLHTLFGDKLCTVATLRETYGEMADCCAKQEPERNECFLQHKDDNPNLPRLVRPEVDVMCTAFHDNEETFLKKYLYEIARRHPYFYAPELLFFAKRYKAAFTECCQAADKAACLLPKLDELRDEGKASSAKQRLKCASLQKFGERAFKAWAVARLSQRFPKAEFAEVSKLVTDLTKVHTECCHGDLLECADDRADLAKYICENQDSISSKLKECCEKPLLEKSHCIAEVENDEMPADLPSLAADFVESKDVCKNYAEAKDVFLGMFLYEYARRHPDYSVVLLLRLAKTYETTLEKCCAAADPHECYAKVFDEFKPLVEEPQNLIKQNCELFEQLGEYKFQNALLVRYTKKVPQVSTPTLVEVSRNLGKVGSKCCKHPEAKRMPCAEDYLSVVLNQLCVLHEKTPVSDRVTKCCTESLVNRRPCFSALEVDETYVPKEFNAETFTFHADICTLSEKERQIKKQTALVELVKHKPKATKEQLKAVMDDFAAFVEKCCKADDKETCFAEEGKKLVAASQAALGLGGGGSGGGGSGGGGSEAQLVESGAEVKKPGDSLKISCKGSGYSFTSYWIGWVRQMPGKGLEWMGIIYPGDSETTYSPAFQGDVTISVDKSISTAYLQWNSLKASDTGIYYCARRRGNYYMDVWGNGTPVTVSSLKSGGGGSGGGGSGGGGSRSTQSALTQPASVSGSPGQSITISCTGTSSDVGGYNYVSWYQQHPGKAPKLMIYDVSNRPSGVSNRFSGSKSGNTASLTISGLQAEDEADYYCSSYTSSSTRHVFGTGTQLTVLGGGGGSGGGGSGGGGSAPASSSTKKTQLQLEHLLLDLQMILNGINNYKNPALTAMLTFAFAMPKKATELKHLQCLEEELKPLEEVLNLAQSKNFHLRPRDLISNINVIVLELKGSETTFMCEYADETATIVEFLNRWITFAQSIISTLT

SEQ ID NO: 17 - protein, 999 aa, Artificial Sequence
  HSA-CSPG4-scFv-MK-14
DAHKSEVAHRFKDLGEENFKALVLIAFAQYLQQCPFEDHVKLVNEVTEFAKTCVADESAENCDKSLHTLFGDKLCTVATLRETYGEMADCCAKQEPERNECFLQHKDDNPNLPRLVRPEVDVMCTAFHDNEETFLKKYLYEIARRHPYFYAPELLFFAKRYKAAFTECCQAADKAACLLPKLDELRDEGKASSAKQRLKCASLQKFGERAFKAWAVARLSQRFPKAEFAEVSKLVTDLTKVHTECCHGDLLECADDRADLAKYICENQDSISSKLKECCEKPLLEKSHCIAEVENDEMPADLPSLAADFVESKDVCKNYAEAKDVFLGMFLYEYARRHPDYSVVLLLRLAKTYETTLEKCCAAADPHECYAKVFDEFKPLVEEPQNLIKQNCELFEQLGEYKFQNALLVRYTKKVPQVSTPTLVEVSRNLGKVGSKCCKHPEAKRMPCAEDYLSVVLNQLCVLHEKTPVSDRVTKCCTESLVNRRPCFSALEVDETYVPKEFNAETFTFHADICTLSEKERQIKKQTALVELVKHKPKATKEQLKAVMDDFAAFVEKCCKADDKETCFAEEGKKLVAASQAALGLGGGGSGGGGSGGGGSEAQLVESGAEVKKPGDSLKISCKGSGYSFTSYWIGWVRQMPGKGLEWMGIIYPGDSETTYSPAFQGDVTISVDKSISTAYLQWNSLKASDTGIYYCARRRGNYYMDVWGNGTPVTVSSLKSGGGGSGGGGSGGGGSRSTQSALTQPASVSGSPGQSITISCTGTSSDVGGYNYVSWYQQHPGKAPKLMIYDVSNRPSGVSNRFSGSKSGNTASLTISGLQAEDEADYYCSSYTSSSTRHVFGTGTQLTVLGGGGGSGGGGSGGGGSAPASSSTKKTQLQLEHLLLDLQMILNGINNYKNPKLTRMLTFKFYMPKKATELKHLQCLEEELKPLEEVLNLAQSKNFHLRPRDLISNINVIVLELKGSETTFMCEYADETATIVEFLNRWITFAQSIISTLT

SEQ ID NO: 18 - protein, 999 aa, Artificial Sequence
  HSA-CSPG4-scFv-MK-15
DAHKSEVAHRFKDLGEENFKALVLIAFAQYLQQCPFEDHVKLVNEVTEFAKTCVADESAENCDKSLHTLFGDKLCTVATLRETYGEMADCCAKQEPERNECFLQHKDDNPNLPRLVRPEVDVMCTAFHDNEETFLKKYLYEIARRHPYFYAPELLFFAKRYKAAFTECCQAADKAACLLPKLDELRDEGKASSAKQRLKCASLQKFGERAFKAWAVARLSQRFPKAEFAEVSKLVTDLTKVHTECCHGDLLECADDRADLAKYICENQDSISSKLKECCEKPLLEKSHCIAEVENDEMPADLPSLAADFVESKDVCKNYAEAKDVFLGMFLYEYARRHPDYSVVLLLRLAKTYETTLEKCCAAADPHECYAKVFDEFKPLVEEPQNLIKQNCELFEQLGEYKFQNALLVRYTKKVPQVSTPTLVEVSRNLGKVGSKCCKHPEAKRMPCAEDYLSVVLNQLCVLHEKTPVSDRVTKCCTESLVNRRPCFSALEVDETYVPKEFNAETFTFHADICTLSEKERQIKKQTALVELVKHKPKATKEQLKAVMDDFAAFVEKCCKADDKETCFAEEGKKLVAASQAALGLGGGGSGGGGSGGGGSEAQLVESGAEVKKPGDSLKISCKGSGYSFTSYWIGWVRQMPGKGLEWMGIIYPGDSETTYSPAFQGDVTISVDKSISTAYLQWNSLKASDTGIYYCARRRGNYYMDVWGNGTPVTVSSLKSGGGGSGGGGSGGGGSRSTQSALTQPASVSGSPGQSITISCTGTSSDVGGYNYVSWYQQHPGKAPKLMIYDVSNRPSGVSNRFSGSKSGNTASLTISGLQAEDEADYYCSSYTSSSTRHVFGTGTQLTVLGGGGGSGGGGSGGGGSAPASSSTKKTQLQLEHLLLDLQMILNGINNYKNPALTAMLTAKFAMPKKATELKHLQCLEEELKPLEEVLNLAQSKNFHLRPRDLISNINVIVLELKGSETTFMCEYADETATIVEFLNRWITFAQSIISTLT

SEQ ID NO: 19 - protein, 998 aa, Artificial Sequence
  MSA-CSPG4-scFv-MK-6
EAHKSEIAHRYNDLGEQHFKGLVLIAFSQYLQKCSYDEHAKLVQEVTDFAKTCVADESAANCDKSLHTLFGDKLCAIPNLRENYGELADCCTKQEPERNECFLQHKDDNPSLPPFERPEAEAMCTSFKENPTTFMGHYLHEVARRHPYFYAPELLYYAEQYNEILTQCCAEADKESCLTPKLDGVKEKALVSSVRQRMKCSSMQKFGERAFKAWAVARLSQTFPNADFAEITKLATDLTKVNKECCHGDLLECADDRAELAKYMCENQATISSKLQTCCDKPLLKKAHCLSEVEHDTMPADLPAIAADFVEDQEVCKNYAEAKDVFLGTFLYEYSRRHPDYSVSLLLRLAKKYEATLEKCCAEANPPACYGTVLAEFQPLVEEPKNLVKTNCDLYEKLGEYGFQNAILVRYTQKAPQVSTPTLVEAARNLGRVGTKCCTLPEDQRLPCVEDYLSAILNRVCLLHEKTPVSEHVTKCCSGSLVERRPCFSALTVDETYVPKEFKAETFTFHSDICTLPEKEKQIKKQTALAELVKHKPKATAEQLKTVMDDFAQFLDTCCKAADKDTCFSTEGPNLVTRCKDALAGGGGSGGGGSGGGGSEAQLVESGAEVKKPGDSLKISCKGSGYSFTSYWIGWVRQMPGKGLEWMGIIYPGDSETTYSPAFQGDVTISVDKSISTAYLQWNSLKASDTGIYYCARRRGNYYMDVWGNGTPVTVSSLKSGGGGSGGGGSGGGGSRSTQSALTQPASVSGSPGQSITISCTGTSSDVGGYNYVSWYQQHPGKAPKLMIYDVSNRPSGVSNRFSGSKSGNTASLTISGLQAEDEADYYCSSYTSSSTRHVFGTGTQLTVLGGGGGSGGGGSGGGGSAPASSSTKKTQLQLEHLLLDLQMILNGINNYKNPALTAMLTFAFAMPKKATELKHLQCLEEELKPLEEVLNLAQSKNFHLRPRDLISNINVIVLELKGSETTFMCEYADETATIVEFLNRWITFAQSIISTLT

SEQ ID NO: 20 - protein, 998 aa, Artificial Sequence
  MSA-CSPG4-scFv-MK-14
EAHKSEIAHRYNDLGEQHFKGLVLIAFSQYLQKCSYDEHAKLVQEVTDFAKTCVADESAANCDKSLHTLFGDKLCAIPNLRENYGELADCCTKQEPERNECFLQHKDDNPSLPPFERPEAEAMCTSFKENPTTFMGHYLHEVARRHPYFYAPELLYYAEQYNEILTQCCAEADKESCLTPKLDGVKEKALVSSVRQRMKCSSMQKFGERAFKAWAVARLSQTFPNADFAEITKLATDLTKVNKECCHGDLLECADDRAELAKYMCENQATISSKLQTCCDKPLLKKAHCLSEVEHDTMPADLPAIAADFVEDQEVCKNYAEAKDVFLGTFLYEYSRRHPDYSVSLLLRLAKKYEATLEKCCAEANPPACYGTVLAEFQPLVEEPKNLVKTNCDLYEKLGEYGFQNAILVRYTQKAPQVSTPTLVEAARNLGRVGTKCCTLPEDQRLPCVEDYLSAILNRVCLLHEKTPVSEHVTKCCSGSLVERRPCFSALTVDETYVPKEFKAETFTFHSDICTLPEKEKQIKKQTALAELVKHKPKATAEQLKTVMDDFAQFLDTCCKAADKDTCFSTEGPNLVTRCKDALAGGGGSGGGGSGGGGSEAQLVESGAEVKKPGDSLKISCKGSGYSFTSYWIGWVRQMPGKGLEWMGIIYPGDSETTYSPAFQGDVTISVDKSISTAYLQWNSLKASDTGIYYCARRRGNYYMDVWGNGTPVTVSSLKSGGGGSGGGGSGGGGSRSTQSALTQPASVSGSPGQSITISCTGTSSDVGGYNYVSWYQQHPGKAPKLMIYDVSNRPSGVSNRFSGSKSGNTASLTISGLQAEDEADYYCSSYTSSSTRHVFGTGTQLTVLGGGGGSGGGGSGGGGSAPASSSTKKTQLQLEHLLLDLQMILNGINNYKNPKLTRMLTFKFYMPKKATELKHLQCLEEELKPLEEVLNLAQSKNFHLRPRDLISNINVIVLELKGSETTFMCEYADETATIVEFLNRWITFAQSIISTLT

SEQ ID NO: 21 - protein, 5 aa, Artificial Sequence
  linker
GGGGS

SEQ ID NO: 22 - protein, 10 aa, Artificial Sequence
  linker
GGGGSGGGGS

SEQ ID NO: 23 - protein, 15 aa, Artificial Sequence
  linker
GGGGSGGGGSGGGGS

SEQ ID NO: 24 - protein, 20 aa, Artificial Sequence
  linker
GGGGSGGGGSGGGGSGGGGS

SEQ ID NO: 25 - protein, 8 aa, Artificial Sequence
  linker
GGGGGGGG

SEQ ID NO: 26 - protein, 6 aa, Artificial Sequence
  linker
GGGGGG

SEQ ID NO: 27 - protein, 15 aa, Artificial Sequence
  linker
EAAAKEAAAKEAAAK

SEQ ID NO: 28 - protein, 4 aa, Artificial Sequence
  linker
EAAK

SEQ ID NO: 29 - protein, 8 aa, Artificial Sequence
  linker
EAAKEAAK

SEQ ID NO: 30 - protein, 12 aa, Artificial Sequence
  linker
EAAKEAAKEAAK

SEQ ID NO: 31 - protein, 46 aa, Artificial Sequence
  linker
AEAAAKEAAAKEAAAKEAAAKALEAEAAAKEAAAKEAAAKEAAAKA

SEQ ID NO: 32 - protein, 12 aa, Artificial Sequence
  linker
AEAAAKEAAAKA

SEQ ID NO: 33 - protein, 5 aa, Artificial Sequence
  linker
PAPAP